European Patent Application EP 4 357 461 A2, published April 24, 2024. Title: DETERMINATION OF BASE MODIFICATIONS OF NUCLEIC ACIDS. Applicant: THE CHINESE UNIVERSITY OF HONG KONG. Application EP. The sequence listing filed with the application follows.

SEQUENCE LISTING (5 sequences)

SEQ ID NO: 1 - RNA, 36 nt, synthetic construct
  misc_feature 1..36: note = Description of Artificial Sequence: Synthetic oligonucleotide
  source 1..36: mol_type = other RNA
gcctgtaatcccagcactttgttttagagctatgct

SEQ ID NO: 2 - RNA, 67 nt, synthetic construct
  misc_feature 1..67: note = Description of Artificial Sequence: Synthetic oligonucleotide
  source 1..67: mol_type = other RNA
agcatagcaagttaaaataaggctagtccgttatcaacttgaaaaagtggcaccgagtcggtgcttt

SEQ ID NO: 3 - RNA, 36 nt, synthetic construct
  misc_feature 1..36: note = Description of Artificial Sequence: Synthetic oligonucleotide
  source 1..36: mol_type = other RNA
agggtctcgctctgtcgcccgttttagagctatgct

SEQ ID NO: 4 - DNA, 10 bp, synthetic construct
  misc_feature 1..10: note = Description of Artificial Sequence: Synthetic oligonucleotide
  source 1..10: mol_type = other DNA
atacgtacgt

SEQ ID NO: 5 - DNA, 10 bp, synthetic construct
  misc_feature 1..10: note = Description of Artificial Sequence: Synthetic oligonucleotide
  source 1..10: mol_type = other DNA
atacgtacgt